European Patent Specification EP 3 294 335 B1, published July 5, 2023. Title: Humanized Affinity-Matured Anti-FcRn Antibodies. Applicant: Syntimmune, Inc. The sequence listing filed with the application follows.

SEQUENCE LISTING (78 sequences)

SEQ ID NO: 1 - DNA, 15 bp, Mus musculus
  CDS (1)..(15)
agctatggtataagc

SEQ ID NO: 2 - protein, 5 aa, Mus musculus
SYGIS

SEQ ID NO: 3 - DNA, 51 bp, Mus musculus
  CDS (1)..(51)
gagatttatcctagaagtggtaatacttactacaatgagaagttcaagggc

SEQ ID NO: 4 - protein, 17 aa, Mus musculus
EIYPRSGNTYYNEKFKG

SEQ ID NO: 5 - DNA, 33 bp, Mus musculus
  CDS (1)..(33)
aaggcaagtgaccacattaataattggttagcc

SEQ ID NO: 6 - protein, 11 aa, Mus musculus
KASDHINNWLA

SEQ ID NO: 7 - DNA, 21 bp, Mus musculus
  CDS (1)..(21)
ggtgcaaccagtttggaaact

SEQ ID NO: 8 - protein, 7 aa, Mus musculus
GATSLET

SEQ ID NO: 9 - DNA, 27 bp, Mus musculus
  CDS (1)..(27)
caacagtattggagtactccgtacacg

SEQ ID NO: 10 - protein, 9 aa, Mus musculus
QQYWSTPYT

SEQ ID NO: 11 - DNA, 354 bp, Artificial Sequence
  humanized
  CDS (1)..(354)
  misc_feature (91)..(105): CDR
  misc_feature (148)..(198): CDR
  misc_feature (295)..(321): CDR
caggttcagctggtgcagtctggagctgagctgaagaagcctggggcttcagtgaagctgtcctgcaaggcttctggctacaccttcacannnnnnnnnnnnnnntgggtgaagcaggccactggacagggccttgagtggattggannnnnnnnnnnnnnnnnnnnnnnnnnnnnnnnnnnnnnnnnnnnnnnnnnnagagccacactgactgcagacaaatccacgagcacagcgtacatggagctccgcagcctgagatctgaggactctgcggtctatttctgtgcaagannnnnnnnnnnnnnnnnnnnnnnnnnncggggcacagggaccacggtcaccgtctcctca

SEQ ID NO: 12 - protein, 118 aa, Artificial Sequence
  misc_feature (31)..(31): The 'Xaa' at location 31 stands for Lys, Asn, Arg, Ser, Thr, Ile, Met, Glu, Asp, Gly, Ala, Val, Gln, His, Pro, Leu, Tyr, Trp, Cys, or Phe.
  misc_feature (32)..(32): The 'Xaa' at location 32 stands for Lys, Asn, Arg, Ser, Thr, Ile, Met, Glu, Asp, Gly, Ala, Val, Gln, His, Pro, Leu, Tyr, Trp, Cys, or Phe.
  misc_feature (33)..(33): The 'Xaa' at location 33 stands for Lys, Asn, Arg, Ser, Thr, Ile, Met, Glu, Asp, Gly, Ala, Val, Gln, His, Pro, Leu, Tyr, Trp, Cys, or Phe.
  misc_feature (34)..(34): The 'Xaa' at location 34 stands for Lys, Asn, Arg, Ser, Thr, Ile, Met, Glu, Asp, Gly, Ala, Val, Gln, His, Pro, Leu, Tyr, Trp, Cys, or Phe.
  misc_feature (35)..(35): The 'Xaa' at location 35 stands for Lys, Asn, Arg, Ser, Thr, Ile, Met, Glu, Asp, Gly, Ala, Val, Gln, His, Pro, Leu, Tyr, Trp, Cys, or Phe.
  misc_feature (50)..(50): The 'Xaa' at location 50 stands for Lys, Asn, Arg, Ser, Thr, Ile, Met, Glu, Asp, Gly, Ala, Val, Gln, His, Pro, Leu, Tyr, Trp, Cys, or Phe.
  misc_feature (51)..(51): The 'Xaa' at location 51 stands for Lys, Asn, Arg, Ser, Thr, Ile, Met, Glu, Asp, Gly, Ala, Val, Gln, His, Pro, Leu, Tyr, Trp, Cys, or Phe.
  misc_feature (52)..(52): The 'Xaa' at location 52 stands for Lys, Asn, Arg, Ser, Thr, Ile, Met, Glu, Asp, Gly, Ala, Val, Gln, His, Pro, Leu, Tyr, Trp, Cys, or Phe.
  misc_feature (53)..(53): The 'Xaa' at location 53 stands for Lys, Asn, Arg, Ser, Thr, Ile, Met, Glu, Asp, Gly, Ala, Val, Gln, His, Pro, Leu, Tyr, Trp, Cys, or Phe.
  misc_feature (54)..(54): The 'Xaa' at location 54 stands for Lys, Asn, Arg, Ser, Thr, Ile, Met, Glu, Asp, Gly, Ala, Val, Gln, His, Pro, Leu, Tyr, Trp, Cys, or Phe.
  misc_feature (55)..(55): The 'Xaa' at location 55 stands for Lys, Asn, Arg, Ser, Thr, Ile, Met, Glu, Asp, Gly, Ala, Val, Gln, His, Pro, Leu, Tyr, Trp, Cys, or Phe.
  misc_feature (56)..(56): The 'Xaa' at location 56 stands for Lys, Asn, Arg, Ser, Thr, Ile, Met, Glu, Asp, Gly, Ala, Val, Gln, His, Pro, Leu, Tyr, Trp, Cys, or Phe.
  misc_feature (57)..(57): The 'Xaa' at location 57 stands for Lys, Asn, Arg, Ser, Thr, Ile, Met, Glu, Asp, Gly, Ala, Val, Gln, His, Pro, Leu, Tyr, Trp, Cys, or Phe.
  misc_feature (58)..(58): The 'Xaa' at location 58 stands for Lys, Asn, Arg, Ser, Thr, Ile, Met, Glu, Asp, Gly, Ala, Val, Gln, His, Pro, Leu, Tyr, Trp, Cys, or Phe.
  misc_feature (59)..(59): The 'Xaa' at location 59 stands for Lys, Asn, Arg, Ser, Thr, Ile, Met, Glu, Asp, Gly, Ala, Val, Gln, His, Pro, Leu, Tyr, Trp, Cys, or Phe.
  misc_feature (60)..(60): The 'Xaa' at location 60 stands for Lys, Asn, Arg, Ser, Thr, Ile, Met, Glu, Asp, Gly, Ala, Val, Gln, His, Pro, Leu, Tyr, Trp, Cys, or Phe.
  misc_feature (61)..(61): The 'Xaa' at location 61 stands for Lys, Asn, Arg, Ser, Thr, Ile, Met, Glu, Asp, Gly, Ala, Val, Gln, His, Pro, Leu, Tyr, Trp, Cys, or Phe.
  misc_feature (62)..(62): The 'Xaa' at location 62 stands for Lys, Asn, Arg, Ser, Thr, Ile, Met, Glu, Asp, Gly, Ala, Val, Gln, His, Pro, Leu, Tyr, Trp, Cys, or Phe.
  misc_feature (63)..(63): The 'Xaa' at location 63 stands for Lys, Asn, Arg, Ser, Thr, Ile, Met, Glu, Asp, Gly, Ala, Val, Gln, His, Pro, Leu, Tyr, Trp, Cys, or Phe.
  misc_feature (64)..(64): The 'Xaa' at location 64 stands for Lys, Asn, Arg, Ser, Thr, Ile, Met, Glu, Asp, Gly, Ala, Val, Gln, His, Pro, Leu, Tyr, Trp, Cys, or Phe.
  misc_feature (65)..(65): The 'Xaa' at location 65 stands for Lys, Asn, Arg, Ser, Thr, Ile, Met, Glu, Asp, Gly, Ala, Val, Gln, His, Pro, Leu, Tyr, Trp, Cys, or Phe.
  misc_feature (66)..(66): The 'Xaa' at location 66 stands for Lys, Asn, Arg, Ser, Thr, Ile, Met, Glu, Asp, Gly, Ala, Val, Gln, His, Pro, Leu, Tyr, Trp, Cys, or Phe.
  misc_feature (99)..(99): The 'Xaa' at location 99 stands for Lys, Asn, Arg, Ser, Thr, Ile, Met, Glu, Asp, Gly, Ala, Val, Gln, His, Pro, Leu, Tyr, Trp, Cys, or Phe.
  misc_feature (100)..(100): The 'Xaa' at location 100 stands for Lys, Asn, Arg, Ser, Thr, Ile, Met, Glu, Asp, Gly, Ala, Val, Gln, His, Pro, Leu, Tyr, Trp, Cys, or Phe.
  misc_feature (101)..(101): The 'Xaa' at location 101 stands for Lys, Asn, Arg, Ser, Thr, Ile, Met, Glu, Asp, Gly, Ala, Val, Gln, His, Pro, Leu, Tyr, Trp, Cys, or Phe.
  misc_feature (102)..(102): The 'Xaa' at location 102 stands for Lys, Asn, Arg, Ser, Thr, Ile, Met, Glu, Asp, Gly, Ala, Val, Gln, His, Pro, Leu, Tyr, Trp, Cys, or Phe.
  misc_feature (103)..(103): The 'Xaa' at location 103 stands for Lys, Asn, Arg, Ser, Thr, Ile, Met, Glu, Asp, Gly, Ala, Val, Gln, His, Pro, Leu, Tyr, Trp, Cys, or Phe.
  misc_feature (104)..(104): The 'Xaa' at location 104 stands for Lys, Asn, Arg, Ser, Thr, Ile, Met, Glu, Asp, Gly, Ala, Val, Gln, His, Pro, Leu, Tyr, Trp, Cys, or Phe.
  misc_feature (105)..(105): The 'Xaa' at location 105 stands for Lys, Asn, Arg, Ser, Thr, Ile, Met, Glu, Asp, Gly, Ala, Val, Gln, His, Pro, Leu, Tyr, Trp, Cys, or Phe.
  misc_feature (106)..(106): The 'Xaa' at location 106 stands for Lys, Asn, Arg, Ser, Thr, Ile, Met, Glu, Asp, Gly, Ala, Val, Gln, His, Pro, Leu, Tyr, Trp, Cys, or Phe.
  misc_feature (107)..(107): The 'Xaa' at location 107 stands for Lys, Asn, Arg, Ser, Thr, Ile, Met, Glu, Asp, Gly, Ala, Val, Gln, His, Pro, Leu, Tyr, Trp, Cys, or Phe.
  Synthetic Construct
QVQLVQSGAELKKPGASVKLSCKASGYTFTXXXXXWVKQATGQGLEWIGXXXXXXXXXXXXXXXXXRATLTADKSTSTAYMELRSLRSEDSAVYFCARXXXXXXXXXRGTGTTVTVSS

SEQ ID NO: 13 - DNA, 354 bp, Artificial Sequence
  humanized
  CDS (1)..(354)
  misc_feature (91)..(105): CDR
  misc_feature (148)..(198): CDR
  misc_feature (295)..(321): CDR
caggttcagctggtgcagtctggagctgaggtgaagaagcctggggcttcagtgaagctgtcctgcaaggcttctggctacaccttcacannnnnnnnnnnnnnntgggtgaagcaggcccctggacagggccttgagtggattggannnnnnnnnnnnnnnnnnnnnnnnnnnnnnnnnnnnnnnnnnnnnnnnnnnagagccacactgactgcagacaaatccacgagcacagcgtacatggagctccgcagcctgagatctgaggacactgcggtctatttctgtgcaagannnnnnnnnnnnnnnnnnnnnnnnnnncggggcacagggaccacggtcaccgtctcctca

SEQ ID NO: 14 - protein, 118 aa, Artificial Sequence
  misc_feature (31)..(31): The 'Xaa' at location 31 stands for Lys, Asn, Arg, Ser, Thr, Ile, Met, Glu, Asp, Gly, Ala, Val, Gln, His, Pro, Leu, Tyr, Trp, Cys, or Phe.
  misc_feature (32)..(32): The 'Xaa' at location 32 stands for Lys, Asn, Arg, Ser, Thr, Ile, Met, Glu, Asp, Gly, Ala, Val, Gln, His, Pro, Leu, Tyr, Trp, Cys, or Phe.
  misc_feature (33)..(33): The 'Xaa' at location 33 stands for Lys, Asn, Arg, Ser, Thr, Ile, Met, Glu, Asp, Gly, Ala, Val, Gln, His, Pro, Leu, Tyr, Trp, Cys, or Phe.
  misc_feature (34)..(34): The 'Xaa' at location 34 stands for Lys, Asn, Arg, Ser, Thr, Ile, Met, Glu, Asp, Gly, Ala, Val, Gln, His, Pro, Leu, Tyr, Trp, Cys, or Phe.
  misc_feature (35)..(35): The 'Xaa' at location 35 stands for Lys, Asn, Arg, Ser, Thr, Ile, Met, Glu, Asp, Gly, Ala, Val, Gln, His, Pro, Leu, Tyr, Trp, Cys, or Phe.
  misc_feature (50)..(50): The 'Xaa' at location 50 stands for Lys, Asn, Arg, Ser, Thr, Ile, Met, Glu, Asp, Gly, Ala, Val, Gln, His, Pro, Leu, Tyr, Trp, Cys, or Phe.
  misc_feature (51)..(51): The 'Xaa' at location 51 stands for Lys, Asn, Arg, Ser, Thr, Ile, Met, Glu, Asp, Gly, Ala, Val, Gln, His, Pro, Leu, Tyr, Trp, Cys, or Phe.
  misc_feature (52)..(52): The 'Xaa' at location 52 stands for Lys, Asn, Arg, Ser, Thr, Ile, Met, Glu, Asp, Gly, Ala, Val, Gln, His, Pro, Leu, Tyr, Trp, Cys, or Phe.
  misc_feature (53)..(53): The 'Xaa' at location 53 stands for Lys, Asn, Arg, Ser, Thr, Ile, Met, Glu, Asp, Gly, Ala, Val, Gln, His, Pro, Leu, Tyr, Trp, Cys, or Phe.
  misc_feature (54)..(54): The 'Xaa' at location 54 stands for Lys, Asn, Arg, Ser, Thr, Ile, Met, Glu, Asp, Gly, Ala, Val, Gln, His, Pro, Leu, Tyr, Trp, Cys, or Phe.
  misc_feature (55)..(55): The 'Xaa' at location 55 stands for Lys, Asn, Arg, Ser, Thr, Ile, Met, Glu, Asp, Gly, Ala, Val, Gln, His, Pro, Leu, Tyr, Trp, Cys, or Phe.
  misc_feature (56)..(56): The 'Xaa' at location 56 stands for Lys, Asn, Arg, Ser, Thr, Ile, Met, Glu, Asp, Gly, Ala, Val, Gln, His, Pro, Leu, Tyr, Trp, Cys, or Phe.
  misc_feature (57)..(57): The 'Xaa' at location 57 stands for Lys, Asn, Arg, Ser, Thr, Ile, Met, Glu, Asp, Gly, Ala, Val, Gln, His, Pro, Leu, Tyr, Trp, Cys, or Phe.
  misc_feature (58)..(58): The 'Xaa' at location 58 stands for Lys, Asn, Arg, Ser, Thr, Ile, Met, Glu, Asp, Gly, Ala, Val, Gln, His, Pro, Leu, Tyr, Trp, Cys, or Phe.
  misc_feature (59)..(59): The 'Xaa' at location 59 stands for Lys, Asn, Arg, Ser, Thr, Ile, Met, Glu, Asp, Gly, Ala, Val, Gln, His, Pro, Leu, Tyr, Trp, Cys, or Phe.
  misc_feature (60)..(60): The 'Xaa' at location 60 stands for Lys, Asn, Arg, Ser, Thr, Ile, Met, Glu, Asp, Gly, Ala, Val, Gln, His, Pro, Leu, Tyr, Trp, Cys, or Phe.
  misc_feature (61)..(61): The 'Xaa' at location 61 stands for Lys, Asn, Arg, Ser, Thr, Ile, Met, Glu, Asp, Gly, Ala, Val, Gln, His, Pro, Leu, Tyr, Trp, Cys, or Phe.
  misc_feature (62)..(62): The 'Xaa' at location 62 stands for Lys, Asn, Arg, Ser, Thr, Ile, Met, Glu, Asp, Gly, Ala, Val, Gln, His, Pro, Leu, Tyr, Trp, Cys, or Phe.
  misc_feature (63)..(63): The 'Xaa' at location 63 stands for Lys, Asn, Arg, Ser, Thr, Ile, Met, Glu, Asp, Gly, Ala, Val, Gln, His, Pro, Leu, Tyr, Trp, Cys, or Phe.
  misc_feature (64)..(64): The 'Xaa' at location 64 stands for Lys, Asn, Arg, Ser, Thr, Ile, Met, Glu, Asp, Gly, Ala, Val, Gln, His, Pro, Leu, Tyr, Trp, Cys, or Phe.
  misc_feature (65)..(65): The 'Xaa' at location 65 stands for Lys, Asn, Arg, Ser, Thr, Ile, Met, Glu, Asp, Gly, Ala, Val, Gln, His, Pro, Leu, Tyr, Trp, Cys, or Phe.
  misc_feature (66)..(66): The 'Xaa' at location 66 stands for Lys, Asn, Arg, Ser, Thr, Ile, Met, Glu, Asp, Gly, Ala, Val, Gln, His, Pro, Leu, Tyr, Trp, Cys, or Phe.
  misc_feature (99)..(99): The 'Xaa' at location 99 stands for Lys, Asn, Arg, Ser, Thr, Ile, Met, Glu, Asp, Gly, Ala, Val, Gln, His, Pro, Leu, Tyr, Trp, Cys, or Phe.
  misc_feature (100)..(100): The 'Xaa' at location 100 stands for Lys, Asn, Arg, Ser, Thr, Ile, Met, Glu, Asp, Gly, Ala, Val, Gln, His, Pro, Leu, Tyr, Trp, Cys, or Phe.
  misc_feature (101)..(101): The 'Xaa' at location 101 stands for Lys, Asn, Arg, Ser, Thr, Ile, Met, Glu, Asp, Gly, Ala, Val, Gln, His, Pro, Leu, Tyr, Trp, Cys, or Phe.
  misc_feature (102)..(102): The 'Xaa' at location 102 stands for Lys, Asn, Arg, Ser, Thr, Ile, Met, Glu, Asp, Gly, Ala, Val, Gln, His, Pro, Leu, Tyr, Trp, Cys, or Phe.
  misc_feature (103)..(103): The 'Xaa' at location 103 stands for Lys, Asn, Arg, Ser, Thr, Ile, Met, Glu, Asp, Gly, Ala, Val, Gln, His, Pro, Leu, Tyr, Trp, Cys, or Phe.
  misc_feature (104)..(104): The 'Xaa' at location 104 stands for Lys, Asn, Arg, Ser, Thr, Ile, Met, Glu, Asp, Gly, Ala, Val, Gln, His, Pro, Leu, Tyr, Trp, Cys, or Phe.
  misc_feature (105)..(105): The 'Xaa' at location 105 stands for Lys, Asn, Arg, Ser, Thr, Ile, Met, Glu, Asp, Gly, Ala, Val, Gln, His, Pro, Leu, Tyr, Trp, Cys, or Phe.
  misc_feature (106)..(106): The 'Xaa' at location 106 stands for Lys, Asn, Arg, Ser, Thr, Ile, Met, Glu, Asp, Gly, Ala, Val, Gln, His, Pro, Leu, Tyr, Trp, Cys, or Phe.
  misc_feature (107)..(107): The 'Xaa' at location 107 stands for Lys, Asn, Arg, Ser, Thr, Ile, Met, Glu, Asp, Gly, Ala, Val, Gln, His, Pro, Leu, Tyr, Trp, Cys, or Phe.
  Synthetic Construct
QVQLVQSGAEVKKPGASVKLSCKASGYTFTXXXXXWVKQAPGQGLEWIGXXXXXXXXXXXXXXXXXRATLTADKSTSTAYMELRSLRSEDTAVYFCARXXXXXXXXXRGTGTTVTVSS

SEQ ID NO: 15 - DNA, 354 bp, Artificial Sequence
  humanized
  CDS (1)..(354)
  misc_feature (91)..(105): CDR
  misc_feature (148)..(198): CDR
  misc_feature (295)..(321): CDR
caggttcagctggtgcagtctggagctgaggtgaagaagcctggggcttcagtgaaggtgtcctgcaaggcttctggctacaccttcacannnnnnnnnnnnnnntgggtgcgacaggcccctggacagggccttgagtggattggannnnnnnnnnnnnnnnnnnnnnnnnnnnnnnnnnnnnnnnnnnnnnnnnnnagagccacaattactgcagacaaatccacgagcacagcgtacatggagctccgcagcctgagatctgaggacactgcggtctattactgtgcaagannnnnnnnnnnnnnnnnnnnnnnnnnncggggcacagggaccacggtcaccgtctcctca

SEQ ID NO: 16 - protein, 118 aa, Artificial Sequence
  misc_feature (31)..(31): The 'Xaa' at location 31 stands for Lys, Asn, Arg, Ser, Thr, Ile, Met, Glu, Asp, Gly, Ala, Val, Gln, His, Pro, Leu, Tyr, Trp, Cys, or Phe.
  misc_feature (32)..(32): The 'Xaa' at location 32 stands for Lys, Asn, Arg, Ser, Thr, Ile, Met, Glu, Asp, Gly, Ala, Val, Gln, His, Pro, Leu, Tyr, Trp, Cys, or Phe.
  misc_feature (33)..(33): The 'Xaa' at location 33 stands for Lys, Asn, Arg, Ser, Thr, Ile, Met, Glu, Asp, Gly, Ala, Val, Gln, His, Pro, Leu, Tyr, Trp, Cys, or Phe.
  misc_feature (34)..(34): The 'Xaa' at location 34 stands for Lys, Asn, Arg, Ser, Thr, Ile, Met, Glu, Asp, Gly, Ala, Val, Gln, His, Pro, Leu, Tyr, Trp, Cys, or Phe.
  misc_feature (35)..(35): The 'Xaa' at location 35 stands for Lys, Asn, Arg, Ser, Thr, Ile, Met, Glu, Asp, Gly, Ala, Val, Gln, His, Pro, Leu, Tyr, Trp, Cys, or Phe.
  misc_feature (50)..(50): The 'Xaa' at location 50 stands for Lys, Asn, Arg, Ser, Thr, Ile, Met, Glu, Asp, Gly, Ala, Val, Gln, His, Pro, Leu, Tyr, Trp, Cys, or Phe.
  misc_feature (51)..(51): The 'Xaa' at location 51 stands for Lys, Asn, Arg, Ser, Thr, Ile, Met, Glu, Asp, Gly, Ala, Val, Gln, His, Pro, Leu, Tyr, Trp, Cys, or Phe.
  misc_feature (52)..(52): The 'Xaa' at location 52 stands for Lys, Asn, Arg, Ser, Thr, Ile, Met, Glu, Asp, Gly, Ala, Val, Gln, His, Pro, Leu, Tyr, Trp, Cys, or Phe.
  misc_feature (53)..(53): The 'Xaa' at location 53 stands for Lys, Asn, Arg, Ser, Thr, Ile, Met, Glu, Asp, Gly, Ala, Val, Gln, His, Pro, Leu, Tyr, Trp, Cys, or Phe.
  misc_feature (54)..(54): The 'Xaa' at location 54 stands for Lys, Asn, Arg, Ser, Thr, Ile, Met, Glu, Asp, Gly, Ala, Val, Gln, His, Pro, Leu, Tyr, Trp, Cys, or Phe.
  misc_feature (55)..(55): The 'Xaa' at location 55 stands for Lys, Asn, Arg, Ser, Thr, Ile, Met, Glu, Asp, Gly, Ala, Val, Gln, His, Pro, Leu, Tyr, Trp, Cys, or Phe.
  misc_feature (56)..(56): The 'Xaa' at location 56 stands for Lys, Asn, Arg, Ser, Thr, Ile, Met, Glu, Asp, Gly, Ala, Val, Gln, His, Pro, Leu, Tyr, Trp, Cys, or Phe.
  misc_feature (57)..(57): The 'Xaa' at location 57 stands for Lys, Asn, Arg, Ser, Thr, Ile, Met, Glu, Asp, Gly, Ala, Val, Gln, His, Pro, Leu, Tyr, Trp, Cys, or Phe.
  misc_feature (58)..(58): The 'Xaa' at location 58 stands for Lys, Asn, Arg, Ser, Thr, Ile, Met, Glu, Asp, Gly, Ala, Val, Gln, His, Pro, Leu, Tyr, Trp, Cys, or Phe.
  misc_feature (59)..(59): The 'Xaa' at location 59 stands for Lys, Asn, Arg, Ser, Thr, Ile, Met, Glu, Asp, Gly, Ala, Val, Gln, His, Pro, Leu, Tyr, Trp, Cys, or Phe.
  misc_feature (60)..(60): The 'Xaa' at location 60 stands for Lys, Asn, Arg, Ser, Thr, Ile, Met, Glu, Asp, Gly, Ala, Val, Gln, His, Pro, Leu, Tyr, Trp, Cys, or Phe.
  misc_feature (61)..(61): The 'Xaa' at location 61 stands for Lys, Asn, Arg, Ser, Thr, Ile, Met, Glu, Asp, Gly, Ala, Val, Gln, His, Pro, Leu, Tyr, Trp, Cys, or Phe.
  misc_feature (62)..(62): The 'Xaa' at location 62 stands for Lys, Asn, Arg, Ser, Thr, Ile, Met, Glu, Asp, Gly, Ala, Val, Gln, His, Pro, Leu, Tyr, Trp, Cys, or Phe.
  misc_feature (63)..(63): The 'Xaa' at location 63 stands for Lys, Asn, Arg, Ser, Thr, Ile, Met, Glu, Asp, Gly, Ala, Val, Gln, His, Pro, Leu, Tyr, Trp, Cys, or Phe.
  misc_feature (64)..(64): The 'Xaa' at location 64 stands for Lys, Asn, Arg, Ser, Thr, Ile, Met, Glu, Asp, Gly, Ala, Val, Gln, His, Pro, Leu, Tyr, Trp, Cys, or Phe.
  misc_feature (65)..(65): The 'Xaa' at location 65 stands for Lys, Asn, Arg, Ser, Thr, Ile, Met, Glu, Asp, Gly, Ala, Val, Gln, His, Pro, Leu, Tyr, Trp, Cys, or Phe.
  misc_feature (66)..(66): The 'Xaa' at location 66 stands for Lys, Asn, Arg, Ser, Thr, Ile, Met, Glu, Asp, Gly, Ala, Val, Gln, His, Pro, Leu, Tyr, Trp, Cys, or Phe.
  misc_feature (99)..(99): The 'Xaa' at location 99 stands for Lys, Asn, Arg, Ser, Thr, Ile, Met, Glu, Asp, Gly, Ala, Val, Gln, His, Pro, Leu, Tyr, Trp, Cys, or Phe.
  misc_feature (100)..(100): The 'Xaa' at location 100 stands for Lys, Asn, Arg, Ser, Thr, Ile, Met, Glu, Asp, Gly, Ala, Val, Gln, His, Pro, Leu, Tyr, Trp, Cys, or Phe.
  misc_feature (101)..(101): The 'Xaa' at location 101 stands for Lys, Asn, Arg, Ser, Thr, Ile, Met, Glu, Asp, Gly, Ala, Val, Gln, His, Pro, Leu, Tyr, Trp, Cys, or Phe.
  misc_feature (102)..(102): The 'Xaa' at location 102 stands for Lys, Asn, Arg, Ser, Thr, Ile, Met, Glu, Asp, Gly, Ala, Val, Gln, His, Pro, Leu, Tyr, Trp, Cys, or Phe.
  misc_feature (103)..(103): The 'Xaa' at location 103 stands for Lys, Asn, Arg, Ser, Thr, Ile, Met, Glu, Asp, Gly, Ala, Val, Gln, His, Pro, Leu, Tyr, Trp, Cys, or Phe.
  misc_feature (104)..(104): The 'Xaa' at location 104 stands for Lys, Asn, Arg, Ser, Thr, Ile, Met, Glu, Asp, Gly, Ala, Val, Gln, His, Pro, Leu, Tyr, Trp, Cys, or Phe.
  misc_feature (105)..(105): The 'Xaa' at location 105 stands for Lys, Asn, Arg, Ser, Thr, Ile, Met, Glu, Asp, Gly, Ala, Val, Gln, His, Pro, Leu, Tyr, Trp, Cys, or Phe.
  misc_feature (106)..(106): The 'Xaa' at location 106 stands for Lys, Asn, Arg, Ser, Thr, Ile, Met, Glu, Asp, Gly, Ala, Val, Gln, His, Pro, Leu, Tyr, Trp, Cys, or Phe.
  misc_feature (107)..(107): The 'Xaa' at location 107 stands for Lys, Asn, Arg, Ser, Thr, Ile, Met, Glu, Asp, Gly, Ala, Val, Gln, His, Pro, Leu, Tyr, Trp, Cys, or Phe.
  Synthetic Construct
QVQLVQSGAEVKKPGASVKVSCKASGYTFTXXXXXWVRQAPGQGLEWIGXXXXXXXXXXXXXXXXXRATITADKSTSTAYMELRSLRSEDTAVYYCARXXXXXXXXXRGTGTTVTVSS

SEQ ID NO: 17 - DNA, 354 bp, Artificial Sequence
  humanized
  CDS (1)..(354)
  misc_feature (91)..(105): CDR
  misc_feature (148)..(198): CDR
  misc_feature (295)..(321): CDR
caggttcagctggtgcagtctggagctgaggtgaagaagcctggggcttcagtgaaggtgtcctgcaaggcttctggctacaccttcacannnnnnnnnnnnnnntgggtgcgacaggcccctggacagggccttgagtggattggannnnnnnnnnnnnnnnnnnnnnnnnnnnnnnnnnnnnnnnnnnnnnnnnnnagagtcacaattactgcagacaaatccacgagcacagcgtacatggagctccgcagcctgagatctgaggacactgcggtctattactgtgcaagannnnnnnnnnnnnnnnnnnnnnnnnnncggggcacagggaccacggtcaccgtctcctca

SEQ ID NO: 18 - protein, 118 aa, Artificial Sequence
  misc_feature (31)..(31): The 'Xaa' at location 31 stands for Lys, Asn, Arg, Ser, Thr, Ile, Met, Glu, Asp, Gly, Ala, Val, Gln, His, Pro, Leu, Tyr, Trp, Cys, or Phe.
  misc_feature (32)..(32): The 'Xaa' at location 32 stands for Lys, Asn, Arg, Ser, Thr, Ile, Met, Glu, Asp, Gly, Ala, Val, Gln, His, Pro, Leu, Tyr, Trp, Cys, or Phe.
  misc_feature (33)..(33): The 'Xaa' at location 33 stands for Lys, Asn, Arg, Ser, Thr, Ile, Met, Glu, Asp, Gly, Ala, Val, Gln, His, Pro, Leu, Tyr, Trp, Cys, or Phe.
  misc_feature (34)..(34): The 'Xaa' at location 34 stands for Lys, Asn, Arg, Ser, Thr, Ile, Met, Glu, Asp, Gly, Ala, Val, Gln, His, Pro, Leu, Tyr, Trp, Cys, or Phe.
  misc_feature (35)..(35): The 'Xaa' at location 35 stands for Lys, Asn, Arg, Ser, Thr, Ile, Met, Glu, Asp, Gly, Ala, Val, Gln, His, Pro, Leu, Tyr, Trp, Cys, or Phe.
  misc_feature (50)..(50): The 'Xaa' at location 50 stands for Lys, Asn, Arg, Ser, Thr, Ile, Met, Glu, Asp, Gly, Ala, Val, Gln, His, Pro, Leu, Tyr, Trp, Cys, or Phe.
  misc_feature (51)..(51): The 'Xaa' at location 51 stands for Lys, Asn, Arg, Ser, Thr, Ile, Met, Glu, Asp, Gly, Ala, Val, Gln, His, Pro, Leu, Tyr, Trp, Cys, or Phe.
  misc_feature (52)..(52): The 'Xaa' at location 52 stands for Lys, Asn, Arg, Ser, Thr, Ile, Met, Glu, Asp, Gly, Ala, Val, Gln, His, Pro, Leu, Tyr, Trp, Cys, or Phe.
  misc_feature (53)..(53): The 'Xaa' at location 53 stands for Lys, Asn, Arg, Ser, Thr, Ile, Met, Glu, Asp, Gly, Ala, Val, Gln, His, Pro, Leu, Tyr, Trp, Cys, or Phe.
  misc_feature (54)..(54): The 'Xaa' at location 54 stands for Lys, Asn, Arg, Ser, Thr, Ile, Met, Glu, Asp, Gly, Ala, Val, Gln, His, Pro, Leu, Tyr, Trp, Cys, or Phe.
  misc_feature (55)..(55): The 'Xaa' at location 55 stands for Lys, Asn, Arg, Ser, Thr, Ile, Met, Glu, Asp, Gly, Ala, Val, Gln, His, Pro, Leu, Tyr, Trp, Cys, or Phe.
  misc_feature (56)..(56): The 'Xaa' at location 56 stands for Lys, Asn, Arg, Ser, Thr, Ile, Met, Glu, Asp, Gly, Ala, Val, Gln, His, Pro, Leu, Tyr, Trp, Cys, or Phe.
  misc_feature (57)..(57): The 'Xaa' at location 57 stands for Lys, Asn, Arg, Ser, Thr, Ile, Met, Glu, Asp, Gly, Ala, Val, Gln, His, Pro, Leu, Tyr, Trp, Cys, or Phe.
  misc_feature (58)..(58): The 'Xaa' at location 58 stands for Lys, Asn, Arg, Ser, Thr, Ile, Met, Glu, Asp, Gly, Ala, Val, Gln, His, Pro, Leu, Tyr, Trp, Cys, or Phe.
  misc_feature (59)..(59): The 'Xaa' at location 59 stands for Lys, Asn, Arg, Ser, Thr, Ile, Met, Glu, Asp, Gly, Ala, Val, Gln, His, Pro, Leu, Tyr, Trp, Cys, or Phe.
  misc_feature (60)..(60): The 'Xaa' at location 60 stands for Lys, Asn, Arg, Ser, Thr, Ile, Met, Glu, Asp, Gly, Ala, Val, Gln, His, Pro, Leu, Tyr, Trp, Cys, or Phe.
  misc_feature (61)..(61): The 'Xaa' at location 61 stands for Lys, Asn, Arg, Ser, Thr, Ile, Met, Glu, Asp, Gly, Ala, Val, Gln, His, Pro, Leu, Tyr, Trp, Cys, or Phe.
  misc_feature (62)..(62): The 'Xaa' at location 62 stands for Lys, Asn, Arg, Ser, Thr, Ile, Met, Glu, Asp, Gly, Ala, Val, Gln, His, Pro, Leu, Tyr, Trp, Cys, or Phe.
  misc_feature (63)..(63): The 'Xaa' at location 63 stands for Lys, Asn, Arg, Ser, Thr, Ile, Met, Glu, Asp, Gly, Ala, Val, Gln, His, Pro, Leu, Tyr, Trp, Cys, or Phe.
  misc_feature (64)..(64): The 'Xaa' at location 64 stands for Lys, Asn, Arg, Ser, Thr, Ile, Met, Glu, Asp, Gly, Ala, Val, Gln, His, Pro, Leu, Tyr, Trp, Cys, or Phe.
  misc_feature (65)..(65): The 'Xaa' at location 65 stands for Lys, Asn, Arg, Ser, Thr, Ile, Met, Glu, Asp, Gly, Ala, Val, Gln, His, Pro, Leu, Tyr, Trp, Cys, or Phe.
  misc_feature (66)..(66): The 'Xaa' at location 66 stands for Lys, Asn, Arg, Ser, Thr, Ile, Met, Glu, Asp, Gly, Ala, Val, Gln, His, Pro, Leu, Tyr, Trp, Cys, or Phe.
  misc_feature (99)..(99): The 'Xaa' at location 99 stands for Lys, Asn, Arg, Ser, Thr, Ile, Met, Glu, Asp, Gly, Ala, Val, Gln, His, Pro, Leu, Tyr, Trp, Cys, or Phe.
  misc_feature (100)..(100): The 'Xaa' at location 100 stands for Lys, Asn, Arg, Ser, Thr, Ile, Met, Glu, Asp, Gly, Ala, Val, Gln, His, Pro, Leu, Tyr, Trp, Cys, or Phe.
  misc_feature (101)..(101): The 'Xaa' at location 101 stands for Lys, Asn, Arg, Ser, Thr, Ile, Met, Glu, Asp, Gly, Ala, Val, Gln, His, Pro, Leu, Tyr, Trp, Cys, or Phe.
  misc_feature (102)..(102): The 'Xaa' at location 102 stands for Lys, Asn, Arg, Ser, Thr, Ile, Met, Glu, Asp, Gly, Ala, Val, Gln, His, Pro, Leu, Tyr, Trp, Cys, or Phe.
  misc_feature (103)..(103): The 'Xaa' at location 103 stands for Lys, Asn, Arg, Ser, Thr, Ile, Met, Glu, Asp, Gly, Ala, Val, Gln, His, Pro, Leu, Tyr, Trp, Cys, or Phe.
  misc_feature (104)..(104): The 'Xaa' at location 104 stands for Lys, Asn, Arg, Ser, Thr, Ile, Met, Glu, Asp, Gly, Ala, Val, Gln, His, Pro, Leu, Tyr, Trp, Cys, or Phe.
  misc_feature (105)..(105): The 'Xaa' at location 105 stands for Lys, Asn, Arg, Ser, Thr, Ile, Met, Glu, Asp, Gly, Ala, Val, Gln, His, Pro, Leu, Tyr, Trp, Cys, or Phe.
  misc_feature (106)..(106): The 'Xaa' at location 106 stands for Lys, Asn, Arg, Ser, Thr, Ile, Met, Glu, Asp, Gly, Ala, Val, Gln, His, Pro, Leu, Tyr, Trp, Cys, or Phe.
  misc_feature (107)..(107): The 'Xaa' at location 107 stands for Lys, Asn, Arg, Ser, Thr, Ile, Met, Glu, Asp, Gly, Ala, Val, Gln, His, Pro, Leu, Tyr, Trp, Cys, or Phe.
  Synthetic Construct
QVQLVQSGAEVKKPGASVKVSCKASGYTFTXXXXXWVRQAPGQGLEWIGXXXXXXXXXXXXXXXXXRVTITADKSTSTAYMELRSLRSEDTAVYYCARXXXXXXXXXRGTGTTVTVSS

SEQ ID NO: 19 - DNA, 321 bp, Artificial Sequence
  humanized
  CDS (1)..(321)
gacatccagatgacacaatctccttcctacttgtctgcatctgtaggagacagagtcaccattacttgcaaggcaagtgaccacattaataattggttagcctggtatcagcagaaaccaggacaggctcctaggctcttaatatctggtgcaaccagtttggaaactggggttccttcaagattcagtggcagtggaactggaaaggattacactctcaccattagcagtcttcagactgaagattttgctacgtattactgtcaacagtattggagtactccgtacacgttcggaggggggaccaaggtggaaataaaa

SEQ ID NO: 20 - protein, 107 aa, Artificial Sequence
  Synthetic Construct
DIQMTQSPSYLSASVGDRVTITCKASDHINNWLAWYQQKPGQAPRLLISGATSLETGVPSRFSGSGTGKDYTLTISSLQTEDFATYYCQQYWSTPYTFGGGTKVEIK

SEQ ID NO: 21 - DNA, 321 bp, Artificial Sequence
  humanized
  CDS (1)..(321)
gacatccagatgacacaatctccttcctccttgtctgcatctgtaggagacagagtcaccattacttgcaaggcaagtgaccacattaataattggttagcctggtatcagcagaaaccaggacaggctcctaggctcttaatatctggtgcaaccagtttggaaactggggttccttcaagattcagtggcagtggaactggaaaggattacactctcaccattagcagtcttcagcctgaagattttgctacgtattactgtcaacagtattggagtactccgtacacgttcggaggggggaccaaggtggaaataaaa

SEQ ID NO: 22 - protein, 107 aa, Artificial Sequence
  Synthetic Construct
DIQMTQSPSSLSASVGDRVTITCKASDHINNWLAWYQQKPGQAPRLLISGATSLETGVPSRFSGSGTGKDYTLTISSLQPEDFATYYCQQYWSTPYTFGGGTKVEIK

SEQ ID NO: 23 - DNA, 321 bp, Artificial Sequence
  humanized
  CDS (1)..(321)
gacatccagatgacacaatctccttcctccttgtctgcatctgtaggagacagagtcaccattacttgcaaggcaagtgaccacattaataattggttagcctggtatcagcagaaaccaggacaggctcctaggctcttaatatctggtgcaaccagtttggaaactggggttccttcaagattcagtggcagtggatctggaaaggatttcactctcaccattagcagtcttcagcctgaagattttgctacgtattactgtcaacagtattggagtactccgtacacgttcggaggggggaccaaggtggaaataaaa

SEQ ID NO: 24 - protein, 107 aa, Artificial Sequence
  Synthetic Construct
DIQMTQSPSSLSASVGDRVTITCKASDHINNWLAWYQQKPGQAPRLLISGATSLETGVPSRFSGSGSGKDFTLTISSLQPEDFATYYCQQYWSTPYTFGGGTKVEIK

SEQ ID NO: 25 - DNA, 321 bp, Artificial Sequence
  humanized
  CDS (1)..(321)
gacatccagatgacacaatctccttcctccttgtctgcatctgtaggagacagagtcaccattacttgcaaggcaagtgaccacattaataattggttagcctggtatcagcagaaaccaggacaggctcctaggctcttaatatctggtgcaaccagtttggaaactggggttccttcaagattcagtggcagtggatctggaacagatttcactctcaccattagcagtcttcagcctgaagattttgctacgtattactgtcaacagtattggagtactccgtacacgttcggaggggggaccaaggtggaaataaaa

SEQ ID NO: 26 - protein, 107 aa, Artificial Sequence
  Synthetic Construct
DIQMTQSPSSLSASVGDRVTITCKASDHINNWLAWYQQKPGQAPRLLISGATSLETGVPSRFSGSGSGTDFTLTISSLQPEDFATYYCQQYWSTPYTFGGGTKVEIK

SEQ ID NO: 27 - protein, 9 aa, affinity matured
STTVSPADF

SEQ ID NO: 28 - protein, 118 aa, Artificial Sequence
  affinity matured
QVQLVQSGAELKKPGASVKLSCKASGYTFTSYGISWVKQATGQGLEWIGEIYPRSGNTYYNEKFKGRATLTADKSTSTAYMELRSLRSEDSAVYFCARSTTVSPADFRGTGTTVTVSS

SEQ ID NO: 29 - protein, 9 aa, Artificial Sequence
  affinity matured
STTVSPPPI

SEQ ID NO: 30 - protein, 118 aa, Artificial Sequence
  affinity matured
QVQLVQSGAELKKPGASVKLSCKASGYTFTSYGISWVKQATGQGLEWIGEIYPRSGNTYYNEKFKGRATLTADKSTSTAYMELRSLRSEDSAVYFCARSTTVSPPPIWGTGTTVTVSS

SEQ ID NO: 31 - protein, 9 aa, Artificial Sequence
  affinity matured
STTVSPPAH

SEQ ID NO: 32 - protein, 118 aa, Artificial Sequence
  affinity matured
QVQLVQSGAELKKPGASVKLSCKASGYTFTSYGISWVKQATGQGLEWIGEIYPRSGNTYYNEKFKGRATLTADKSTSTAYMELRSLKSEDSAVYFCARSTTVSPPAHWGTGTTVTVSS

SEQ ID NO: 33 - protein, 9 aa, Artificial Sequence
  affinity matured
STTVAPPRL

SEQ ID NO: 34 - protein, 118 aa, Artificial Sequence
  affinity matured
QVQLVQSGAELKKPGASVKLSCKASGYTFTSYGISWVKQATGQGLEWIGEIYPRSGNTYYNEKFKGRATLTADKSTSTAYMELRSLRSEDSAVYFCARSTTVAPPRLWGTGTTVTVSS

SEQ ID NO: 35 - protein, 9 aa, Artificial Sequence
  affinity matured
STTVHPDRN

SEQ ID NO: 36 - protein, 118 aa, Artificial Sequence
  affinity matured
QVQLVQSGAELKKPGASVKLSCKASGYTFTSYGISWVKQATGQGLEWIGEIYPRSGNTYYNEKFKGRATLTADKSTSTAYMELRSLRSEDSAVYFCARSTTVHPDRNWGTGTTVTVSS

SEQ ID NO: 37 - protein, 9 aa, Artificial Sequence
  affinity matured
STTVSPPAL

SEQ ID NO: 38 - protein, 118 aa, Artificial Sequence
  affinity matured
QVQLVQSGAELKKPGASVKLSCKASGYTFTSYGISWVKQATGQGLEWIGEIYPRSGNTYYNEKFKGRATLTADKSTSTAYMELRSLRSEDSAVYFCARSTTVSPPALWGTGTTVTVSS

SEQ ID NO: 39 - protein, 9 aa, Artificial Sequence
  affinity matured
STTVHPDHN

SEQ ID NO: 40 - protein, 118 aa, Artificial Sequence
  affinity matured
QVQLVQSGAELKKPGASVKLSCKASGYTFTSYGISWVKQATGQGLEWIGEIYPRSGNTYYNEKFKGRATLTADKSTSTAYMELRSLRSEDSAVYFCARSTTVHPDHNWGTGTTVTVSS

SEQ ID NO: 41 - protein, 9 aa, Artificial Sequence
  affinity matured
STTVSPPHL

SEQ ID NO: 42 - protein, 118 aa, Artificial Sequence
  affinity matured
QVQLVQSGAEPKKPGASVKLSCKASGYTFTSYGISWVKQATGQGLEWIGEIYPRSGNTYYNEKFKGRATLTADKSTSTAYMELRSLRSEDSAVYFCARSTTVSPPHLWGTGTTVTVSS

SEQ ID NO: 43 - protein, 9 aa, Artificial Sequence
  affinity matured
STTVAPPPL

SEQ ID NO: 44 - protein, 118 aa, Artificial Sequence
  affinity matured
QVQLVQSGAELKKPGASVKLSCKASGYTFTSYGISWVKQATGQGLEWIGEIYPRSGNTYYNEKFKGRATLTADKSTSTAYMELRSLRSEDSAVYFCARSTTVAPPPLWGTGTTVTVSS

SEQ ID NO: 45 - protein, 9 aa, Artificial Sequence
  affinity matured
STTVSPPHL

SEQ ID NO: 46 - protein, 118 aa, Artificial Sequence
  affinity matured
QVQLVQSGAELKKPGASVKLSCKASGYTFTSYGISWVKQATGQGLEWIGEIYPRSGNTYYNEKFKGRATLTADKSTSTAYMELRSLRSEDSAVYFCARSTTVSPPHLWGTGTTVTVSS

SEQ ID NO: 47 - protein, 9 aa, Artificial Sequence
  affinity matured
STTVAPPGH

SEQ ID NO: 48 - protein, 118 aa, Artificial Sequence
  affinity matured
QVQLVQSGAELKKPGASVKLSCKASGYTFTSYGISWVKQATGQGLEWIGEIYPRSGNTYYNEKFKGRATLTADKSTSTAYMELRSLRSEDSAVYFCARSTTVAPPGHWGTGTTVTVSS

SEQ ID NO: 49 - protein, 9 aa, Artificial Sequence
  affinity matured
STTVSPPRV

SEQ ID NO: 50 - protein, 118 aa, Artificial Sequence
  affinity matured
QVQLVQSGAELKKPGASVKLSCKASGYTFTSYGISWVKQATGQGLEWIGEIYPRSGNTYYNEKFKGRATLTADKSTSTAYMELRSLRSEDSAVYFCARSTTVSPPRVWGTGTTVTVSS

SEQ ID NO: 51 - protein, 9 aa, Artificial Sequence
  affinity matured
STTVSPPPL

SEQ ID NO: 52 - protein, 118 aa, Artificial Sequence
  affinity matured
QVQLVQSGAELKKPGASVKLSCKASGYTFTSYGISWVKQATGQGLEWIGEIYPRSGNTYYNEKFKGRATLTADKSTSTAYMELRSLRSEDSAVYFCARSTTVSPPPLWGTGTTVTVSS

SEQ ID NO: 53 - protein, 9 aa, Artificial Sequence
  affinity matured
STTVAPPAH

SEQ ID NO: 54 - protein, 118 aa, Artificial Sequence
  affinity matured
QVQLVQSGAELKKPGASVKLSCKASGYTFTSYGISWVKQATGQGLEWIGEIYPRSGNTYYNEKFKGRATLTADKSTSTAYMELRSLRSEDSAVYFCARSTTVAPPAHWGTGTTVTVSS

SEQ ID NO: 55 - protein, 9 aa, Artificial Sequence
  affinity matured
STTVRPPGI

SEQ ID NO: 56 - protein, 118 aa, Artificial Sequence
  affinity matured
QVQLVQSGAELKKPGASVKLSCKASGYTFTSYGISWVKQATGQGLEWIGEIYPRSGNTYYNEKFKGRATLTADKSTSTAYMELRSLRSEDSAVYFCARSTTVRPPGIWGTGTTVTVSS

SEQ ID NO: 57 - protein, 9 aa, Artificial Sequence
  affinity matured
STTVSAPGV

SEQ ID NO: 58 - protein, 118 aa, Artificial Sequence
  affinity matured
QVQLVQSGAELKKPGASVKLSCKASGYTFTSYGISWVKQATGQGLEWIGEIYPRSGNTYYNEKFKGRATLTADKSTSTAYMELRSLRSEDSAVYFCARSTTVSAPGVWGTGTTVTVSS

SEQ ID NO: 59 - protein, 9 aa, Artificial Sequence
  affinity matured
NTYGNNPHT

SEQ ID NO: 60 - protein, 107 aa, Artificial Sequence
  affinity matured
DIQMTQSPSYLSASVGDRVTITCKASDHINNWLAWYQQKPGQAPRLLISGATSLETGVPSRFSGSGTGKDYTLTISSLQTEDFATYYCNTYGNNPHTFGGGTKVEIK

SEQ ID NO: 61 - protein, 107 aa, Artificial Sequence
  affinity matured
DIQMTQSPSSLSASVGDRVTITCKASDHINNWLAWYQQKPGQAPRLLISGATSLETGVPSRFSGSGTGKDYTLTISSLQTEDFATYYCNTYGNNPHTFGGGTKVEIK

SEQ ID NO: 62 - protein, 9 aa, Artificial Sequence
  affinity matured
HQYYNTPYT

SEQ ID NO: 63 - protein, 107 aa, Artificial Sequence
  affinity matured
DIQMTQSPSYLSASVGDRVTITCKASDHINNWLAWYQQKPGQAPRLLISGATSLETGVPSRFSGSGTGKDYTLTISSLQTEDFATYYCHQYYNTPYTFGGGTKVEIK

SEQ ID NO: 64 - protein, 107 aa, Artificial Sequence
  affinity matured
DIQMTQSPSSLSASVGDRVTITCKASDHINNWLAWYQQKPGQAPRLLISGATSLETGVPSRFSGSGTGKDYTLTISSLQTEDFATYYCHQYYNTPYTFGGGTKVEIK

SEQ ID NO: 65 - protein, 9 aa, Artificial Sequence
  affinity matured
HQYYSTPYT

SEQ ID NO: 66 - protein, 107 aa, Artificial Sequence
  affinity matured
DIQMTQSPSYLSASVGDRVTITCKASDHINNWLAWYQQKPGQAPRLLISGATSLETGVPSRFSGSGTGKDYTLTISSLQTEDFATYYCHQYYSTPYTFGGGTKVEIK

SEQ ID NO: 67 - protein, 107 aa, Artificial Sequence
  affinity matured
DIQMTQSPSSLSASVGDRVTITCKASDHINNWLAWYQQKPGQAPRLLISGATSLETGVPSRFSGSGTGKDYTLTISSLQTEDFATYYCHQYYSTPYTFGGGTKVEIK

SEQ ID NO: 68 - protein, 9 aa, Artificial Sequence
  affinity matured
QQYYSTPYT

SEQ ID NO: 69 - protein, 107 aa, Artificial Sequence
  affinity matured
DIQMTQSPSYLSASVGDRVTITCKASDHINNWLAWYQQKPGQAPRLLISGATSLETGVPSRFSGSGTGKDYTLTISSLQTEDFATYYCQQYYSTPYTFGGGTKVEIK

SEQ ID NO: 70 - protein, 107 aa, Artificial Sequence
  affinity matured
DIQMTQSPSSLSASVGDRVTITCKASDHINNWLAWYQQKPGQAPRLLISGATSLETGVPSRFSGSGTGKDYTLTISSLQTEDFATYYCQQYYSTPYTFGGGTKVEIK

SEQ ID NO: 71 - DNA, 21 bp, Artificial Sequence
  synthetic sequence
  misc_feature (2)..(2): n is a, c, g, or t
  misc_feature (4)..(5): n is a, c, g, or t
  misc_feature (7)..(8): n is a, c, g, or t
  misc_feature (10)..(11): n is a, c, g, or t
  misc_feature (16)..(16): n is a, c, g, or t
kncnncnncnncsvcnwcygg

SEQ ID NO: 72 - DNA, 33 bp, Artificial Sequence
  synthetic sequence
tgtmrsvmgtvskrsrrcwmcyycbwcrycttc

SEQ ID NO: 73 - protein, 6 aa, Artificial Sequence
  consensus
  VARIANT (2)..(2): residue is A R or S
  VARIANT (5)..(5): residue is G or R
  VARIANT (6)..(6): residue is I L or V
VXPPXX

SEQ ID NO: 74 - protein, 9 aa, Artificial Sequence
  consensus
  VARIANT (5)..(5): residue is A or R or S
  VARIANT (8)..(8): residue is G or R
  VARIANT (9)..(9): residue is I L or V
STTVXPPXX

SEQ ID NO: 75 - protein, 6 aa, Artificial Sequence
  consensus
  VARIANT (2)..(2): residue is A R or S
  VARIANT (5)..(5): residue is A G H P or R
  VARIANT (6)..(6): residue is H I L or V
VXPPXX

SEQ ID NO: 76 - protein, 9 aa, Artificial Sequence
  consensus
  VARIANT (5)..(5): residue is A R or S
  VARIANT (8)..(8): residue is A G H P or R
  VARIANT (9)..(9): residue is H I L or V
STTVXPPXX

SEQ ID NO: 77 - protein, 6 aa, Artificial Sequence
  consensus
  VARIANT (2)..(2): residue is A H R or S
  VARIANT (3)..(3): residue is A or P
  VARIANT (3)..(4): at least one of 3 and 4 is P
  VARIANT (4)..(4): residue is A D or P
  VARIANT (5)..(5): residue is A D G H P or R
  VARIANT (6)..(6): residue is H I L or V
  VARIANT (6)..(6): residue is F H I L N or V
VXXXXX

SEQ ID NO: 78 - protein, 9 aa, Artificial Sequence
  consensus
  VARIANT (5)..(5): residue is A H R or S
  VARIANT (6)..(6): residue is A or P
  VARIANT (6)..(7): at least one of 6 and 7 is P
  VARIANT (7)..(7): residue is A D or P
  VARIANT (8)..(8): residue is A D G H or P
  VARIANT (9)..(9): residue is F H I L N or V
STTVXXXXX